European Patent Specification EP 3 849 558 B1, published June 5, 2024. Title: THIOCARBAMATE DERIVATIVES AS A2A INHIBITORS, PHARMACEUTICAL COMPOSITION THEREOF AND COMBINATIONS WITH ANTICANCER AGENTS. Applicant: ITEOS THERAPEUTICS S.A. The sequence listing filed with the application follows.

SEQUENCE LISTING (6 sequences)

SEQ ID NO: 1 - protein, 9 aa, Artificial Sequence
  HCDR1
YTFTSYYMH

SEQ ID NO: 2 - protein, 17 aa, Artificial Sequence
  HCDR2
VIGPSGASTSYAQKFQG

SEQ ID NO: 3 - protein, 14 aa, Artificial Sequence
  HCDR3
ARDHSDYWSGIMEV

SEQ ID NO: 4 - protein, 12 aa, Artificial Sequence
  LCDR1
RASQSVRSSYLA

SEQ ID NO: 5 - protein, 7 aa, Artificial Sequence
  LCDR2
GASSRAT

SEQ ID NO: 6 - protein, 9 aa, Artificial Sequence
  LCDR3
QQYFSPPWT